European Patent Specification EP 4 017 871 B1, published January 17, 2024. Title: ADENO-ASSOCIATED VIRUS VECTOR DELIVERY OF ALPHA-SARCOGLYCAN AND THE TREATMENT OF MUSCULAR DYSTROPHY. Applicant: Research Institute at Nationwide Children's Hospital. The sequence listing filed with the application follows.

SEQUENCE LISTING (11 sequences)

SEQ ID NO: 1 - DNA, 1164 bp, Homo Sapiens
atggccgagacactgttctggactcctctgctggtggtgctgctggctggactgggagataccgaggctcagcagaccacactgcacccactggtgggccgggtgttcgtgcacaccctggaccatgagacatttctgagtctgccagaacacgtggctgtgccacctgctgtgcatatcacttaccacgcccatctgcagggccatcctgatctgccacggtggctgagatacacccagagatcaccccaccatcctggattcctgtatggaagcgctaccccagaggacaggggactgcaggtgatcgaagtgacagcttacaaccgcgacagttttgatactaccaggcagcgcctggtgctggagattggggatccagaaggacccctgctgccttatcaggccgagttcctggtgcggtcacacgacgctgaggaagtgctgccatcaacacccgccagcagatttctgtccgctctgggaggactgtgggagccaggagaactgcagctgctgaatgtgactagcgctctggataggggaggaagggtgccactgccaatcgagggaaggaaggaaggggtgtacattaaagtgggaagcgcttccccattctccacctgcctgaagatggtggcttctcctgatagtcacgctaggtgcgctcagggacagccaccactgctgtcctgttatgacacactggccccccattttcgcgtggactggtgcaacgtgactctggtggataaatctgtgcctgagccagctgacgaagtgccaacccctggagacggaatcctggagcacgatcctttcttttgtcctccaacagaagccccagacagggatttcctggtggacgctctggtgactctgctggtgcctctgctggtggctctgctgctgaccctgctgctggcttatgtgatgtgctgtcggagagagggacggctgaagagagacctggccacatctgatatccagatggtgcaccattgtactattcacggcaacaccgaggaactgcgccagatggctgcttctagggaggtgccaaggccactgagtacactgcctatgtttaatgtgcacactggcgaacggctgccccctagagtggatagcgcccaggtgccactgattctggaccagcattga

SEQ ID NO: 2 - protein, 387 aa, Homo Sapiens
MAETLFWTPLLVVLLAGLGDTEAQQTTLHPLVGRVFVHTLDHETFLSLPEHVAVPPAVHITYHAHLQGHPDLPRWLRYTQRSPHHPGFLYGSATPEDRGLQVIEVTAYNRDSFDTTRQRLVLEIGDPEGPLLPYQAEFLVRSHDAEEVLPSTPASRFLSALGGLWEPGELQLLNVTSALDRGGRVPLPIEGRKEGVYIKVGSASPFSTCLKMVASPDSHARCAQGQPPLLSCYDTLAPHFRVDWCNVTLVDKSVPEPADEVPTPGDGILEHDPFFCPPTEAPDRDFLVDALVTLLVPLLVALLLTLLLAYVMCCRREGRLKRDLATSDIQMVHHCTIHGNTEELRQMAASREVPRPLSTLPMFNVHTGERLPPRVDSAQVPLILDQH

SEQ ID NO: 3 - DNA, 714 bp, Artificial Sequence
  Synthetic Polypeptide
ccactacgggtctaggctgcccatgtaaggaggcaaggcctggggacacccgagatgcctggttataattaaccccaacacctgctgcccccccccccccaacacctgctgcctgagcctgagcggttaccccaccccggtgcctgggtcttaggctctgtacaccatggaggagaagctcgctctaaaaataaccctgtccctggtggatccactacgggtctatgctgcccatgtaaggaggcaaggcctggggacacccgagatgcctggttataattaaccccaacacctgctgcccccccccccccaacacctgctgcctgagcctgagcggttaccccaccccggtgcctgggtcttaggctctgtacaccatggaggagaagctcgctctaaaaataaccctgtccctggtggaccactacgggtctaggctgcccatgtaaggaggcaaggcctggggacacccgagatgcctggttataattaaccccaacacctgctgccccccccccccaacacctgctgcctgagcctgagcggttaccccaccccggtgcctgggtcttaggctctgtacaccatggaggagaagctcgctctaaaaataaccctgtccctggtcctccctggggacagcccctcctggctagtcacaccctgtaggctcctctatataacccaggggcacaggggctgcccccgggtcac

SEQ ID NO: 4 - DNA, 2476 bp, Artificial Sequence
  Synthetic Polypeptide
ctgcgcgctcgctcgctcactgaggccgcccgggcaaagcccgggcgtcgggcgacctttggtcgcccggcctcagtgagcgagcgagcgcgcagagagggagtggggttaaccaattggcggccgcaaacttgcatgccccactacgggtctaggctgcccatgtaaggaggcaaggcctggggacacccgagatgcctggttataattaaccccaacacctgctgcccccccccccccaacacctgctgcctgagcctgagcggttaccccaccccggtgcctgggtcttaggctctgtacaccatggaggagaagctcgctctaaaaataaccctgtccctggtggatccactacgggtctatgctgcccatgtaaggaggcaaggcctggggacacccgagatgcctggttataattaaccccaacacctgctgcccccccccccccaacacctgctgcctgagcctgagcggttaccccaccccggtgcctgggtcttaggctctgtacaccatggaggagaagctcgctctaaaaataaccctgtccctggtggaccactacgggtctaggctgcccatgtaaggaggcaaggcctggggacacccgagatgcctggttataattaaccccaacacctgctgccccccccccccaacacctgctgcctgagcctgagcggttaccccaccccggtgcctgggtcttaggctctgtacaccatggaggagaagctcgctctaaaaataaccctgtccctggtcctccctggggacagcccctcctggctagtcacaccctgtaggctcctctatataacccaggggcacaggggctgcccccgggtcacctgcagaagttggtcgtgaggcactgggcaggtaagtatcaaggttacaagacaggtttaaggagaccaatagaaactgggcttgtcgagacagagaagactcttgcgtttctgataggcacctattggtcttactgacatccactttgcctttctctccacaggtgtccactcccagttcaattacagcgcgtggtaccaccatggccgagacactgttctggactcctctgctggtggtgctgctggctggactgggagataccgaggctcagcagaccacactgcacccactggtgggccgggtgttcgtgcacaccctggaccatgagacatttctgagtctgccagaacacgtggctgtgccacctgctgtgcatatcacttaccacgcccatctgcagggccatcctgatctgccacggtggctgagatacacccagagatcaccccaccatcctggattcctgtatggaagcgctaccccagaggacaggggactgcaggtgatcgaagtgacagcttacaaccgcgacagttttgatactaccaggcagcgcctggtgctggagattggggatccagaaggacccctgctgccttatcaggccgagttcctggtgcggtcacacgacgctgaggaagtgctgccatcaacacccgccagcagatttctgtccgctctgggaggactgtgggagccaggagaactgcagctgctgaatgtgactagcgctctggataggggaggaagggtgccactgccaatcgagggaaggaaggaaggggtgtacattaaagtgggaagcgcttccccattctccacctgcctgaagatggtggcttctcctgatagtcacgctaggtgcgctcagggacagccaccactgctgtcctgttatgacacactggccccccattttcgcgtggactggtgcaacgtgactctggtggataaatctgtgcctgagccagctgacgaagtgccaacccctggagacggaatcctggagcacgatcctttcttttgtcctccaacagaagccccagacagggatttcctggtggacgctctggtgactctgctggtgcctctgctggtggctctgctgctgaccctgctgctggcttatgtgatgtgctgtcggagagagggacggctgaagagagacctggccacatctgatatccagatggtgcaccattgtactattcacggcaacaccgaggaactgcgccagatggctgcttctagggaggtgccaaggccactgagtacactgcctatgtttaatgtgcacactggcgaacggctgccccctagagtggatagcgcccaggtgccactgattctggaccagcattgaggccgcaataaaagatctttattttcattagatctgtgtgttggttttttgtgtgtcctgcaggggcgcgcctctagagcatggctacgtagataagtagcatggcgggttaatcattaactacaaggaacccctagtgatggagttggccactccctctctgcgcgctcgctcgctcactgaggccgggcgaccaaaggtcgcccgacgcccgggctttgcccgggcggcctcagtgagcgagcgagcgcgcag

SEQ ID NO: 5 - DNA, 110 bp, Artificial Sequence
  Synthetic Polypeptide
ctgcgcgctcgctcgctcactgaggccgcccgggcaaagcccgggcgtcgggcgacctttggtcgcccggcctcagtgagcgagcgagcgcgcagagagggagtggggtt

SEQ ID NO: 6 - DNA, 104 bp, Artificial Sequence
  Synthetic Polypeptide
ccactccctctctgcgcgctcgctcgctcactgaggccgggcgaccaaaggtcgcccgacgcccgggctttgcccgggcggcctcagtgagcgagcgagcgcgc

SEQ ID NO: 7 - DNA, 53 bp, Artificial Sequence
  Synthetic Polypeptide
ggccgcaataaaagatctttattttcattagatctgtgtgttggttttttgtg

SEQ ID NO: 8 - DNA, 5749 bp, Artificial Sequence
  Synthetic Polypeptide
atgcagctgcgcgctcgctcgctcactgaggccgcccgggcaaagcccgggcgtcgggcgacctttggtcgcccggcctcagtgagcgagcgagcgcgcagagagggagtggggttaaccaattggcggccgcaaacttgcatgccccactacgggtctaggctgcccatgtaaggaggcaaggcctggggacacccgagatgcctggttataattaaccccaacacctgctgcccccccccccccaacacctgctgcctgagcctgagcggttaccccaccccggtgcctgggtcttaggctctgtacaccatggaggagaagctcgctctaaaaataaccctgtccctggtggatccactacgggtctatgctgcccatgtaaggaggcaaggcctggggacacccgagatgcctggttataattaaccccaacacctgctgcccccccccccccaacacctgctgcctgagcctgagcggttaccccaccccggtgcctgggtcttaggctctgtacaccatggaggagaagctcgctctaaaaataaccctgtccctggtggaccactacgggtctaggctgcccatgtaaggaggcaaggcctggggacacccgagatgcctggttataattaaccccaacacctgctgccccccccccccaacacctgctgcctgagcctgagcggttaccccaccccggtgcctgggtcttaggctctgtacaccatggaggagaagctcgctctaaaaataaccctgtccctggtcctccctggggacagcccctcctggctagtcacaccctgtaggctcctctatataacccaggggcacaggggctgcccccgggtcacctgcagaagttggtcgtgaggcactgggcaggtaagtatcaaggttacaagacaggtttaaggagaccaatagaaactgggcttgtcgagacagagaagactcttgcgtttctgataggcacctattggtcttactgacatccactttgcctttctctccacaggtgtccactcccagttcaattacagcgcgtggtaccaccatggccgagacactgttctggactcctctgctggtggtgctgctggctggactgggagataccgaggctcagcagaccacactgcacccactggtgggccgggtgttcgtgcacaccctggaccatgagacatttctgagtctgccagaacacgtggctgtgccacctgctgtgcatatcacttaccacgcccatctgcagggccatcctgatctgccacggtggctgagatacacccagagatcaccccaccatcctggattcctgtatggaagcgctaccccagaggacaggggactgcaggtgatcgaagtgacagcttacaaccgcgacagttttgatactaccaggcagcgcctggtgctggagattggggatccagaaggacccctgctgccttatcaggccgagttcctggtgcggtcacacgacgctgaggaagtgctgccatcaacacccgccagcagatttctgtccgctctgggaggactgtgggagccaggagaactgcagctgctgaatgtgactagcgctctggataggggaggaagggtgccactgccaatcgagggaaggaaggaaggggtgtacattaaagtgggaagcgcttccccattctccacctgcctgaagatggtggcttctcctgatagtcacgctaggtgcgctcagggacagccaccactgctgtcctgttatgacacactggccccccattttcgcgtggactggtgcaacgtgactctggtggataaatctgtgcctgagccagctgacgaagtgccaacccctggagacggaatcctggagcacgatcctttcttttgtcctccaacagaagccccagacagggatttcctggtggacgctctggtgactctgctggtgcctctgctggtggctctgctgctgaccctgctgctggcttatgtgatgtgctgtcggagagagggacggctgaagagagacctggccacatctgatatccagatggtgcaccattgtactattcacggcaacaccgaggaactgcgccagatggctgcttctagggaggtgccaaggccactgagtacactgcctatgtttaatgtgcacactggcgaacggctgccccctagagtggatagcgcccaggtgccactgattctggaccagcattgaggccgcaataaaagatctttattttcattagatctgtgtgttggttttttgtgtgtcctgcaggggcgcgcctctagagcatggctacgtagataagtagcatggcgggttaatcattaactacaaggaacccctagtgatggagttggccactccctctctgcgcgctcgctcgctcactgaggccgggcgaccaaaggtcgcccgacgcccgggctttgcccgggcggcctcagtgagcgagcgagcgcgcagctggcgtaatagcgaagaggcccgcaccgatcgcccttcccaacagttgcgcagcctgaatggcgaatggcgattccgttgcaatggctggcggtaatattgttctggatattaccagcaaggccgatagtttgagttcttctactcaggcaagtgatgttattactaatcaaagaagtattgcgacaacggttaatttgcgtgatggacagactcttttactcggtggcctcactgattataaaaacacttctcaggattctggcgtaccgttcctgtctaaaatccctttaatcggcctcctgtttagctcccgctctgattctaacgaggaaagcacgttatacgtgctcgtcaaagcaaccatagtacgcgccctgtagcggcgcattaagcgcggcgggtgtggtggttacgcgcagcgtgaccgctacacttgccagcgccctagcgcccgctcctttcgctttcttcccttcctttctcgccacgttcgccatcttcaaatatgtatccgctcatgagacaataaccctgataaatgcttcaataatattgaaaaaggaagagtcctgaggcggaaagaaccagctgtggaatgtgtgtcagttagggtgtggaaagtccccaggctccccagcaggcagaagtatgcaaagcatgcatctcaattagtcagcaaccaggtgtggaaagtccccaggctccccagcaggcagaagtatgcaaagcatgcatctcaattagtcagcaaccatagtcccgcccctaactccgccccatggctgactaattttttttatttatgcagaggccgaggccgcctcggcctctgagctattccagaagtagtgaggaggcttttttggaggcctaggcttttgcaaagatcgatcaagagacaggatgaggatcgtttcgcatgattgaacaagatggattgcacgcaggttctccggccgcttgggtggagaggctattcggctatgactgggcacaacagacaatcggctgctctgatgccgccgtgttccggctgtcagcgcaggggcgcccggttctttttgtcaagaccgacctgtccggtgccctgaatgaactgcaagacgaggcagcgcggctatcgtggctggccacgacgggcgttccttgcgcagctgtgctcgacgttgtcactgaagcgggaagggactggctgctattgggcgaagtgccggggcaggatctcctgtcatctcaccttgctcctgccgagaaagtatccatcatggctgatgcaatgcggcggctgcatacgcttgatccggctacctgcccattcgaccaccaagcgaaacatcgcatcgagcgagcacgtactcggatggaagccggtcttgtcgatcaggatgatctggacgaagagcatcaggggctcgcgccagccgaactgttcgccaggctcaaggcgagcatgcccgacggcgaggatctcgtcgtgacccatggcgatgcctgcttgccgaatatcatggtggaaaatggccgcttttctggattcatcgactgtggccggctgggtgtggcggaccgctatcaggacatagcgttggctacccgtgatattgctgaagagcttggcggcgaatgggctgaccgcttcctcgtgctttacggtatcgccgctcccgattcgcagcgcatcgccttctatcgccttcttgacgagttcttctgagcgggactctggggttcgaaatgaccgaccaagcgacgcccaacctgccatcacgagatttcgattccaccgccgccttctatgaaaggttgggcttcggaatcgttttccgggacgccggctggatgatcctccagcgcggggatctcatgctggagttcttcgcccaccctagggggaggctaactgaaacacggaaggagacaataccggaaggaacccgcgctatgacggcaataaaaagacagaataaaaacgttgcgcaaactattaactggcgaactacttactctagcttcccggcaacaattaatagactggatggaggcggataaagttgcaggaccacttctgcgctcggcccttccggctggctggtttattgctgataaatctggagccggtgagcgtgggtctcgcggtatcattgcagcactggggccagatggtaagccctcccgtatcgtagttatctacacgacggggagtcaggcaactatggatgaacgaaatagacagatcgctgagataggtgcctcactgattaagcattggtaactgtcagaccaagtttactcatatatactttagattgatttaaaacttcatttttaatttaaaaggatctaggtgaagatcctttttgataatctcatgaccaaaatcccttaacgtgagttttcgttccactgagcgtcagaccccgtagaaaagatcaaaggatcttcttgagatcctttttttctgcgcgtaatctgctgcttgcaaacaaaaaaaccaccgctaccagcggtggtttgtttgccggatcaagagctaccaactctttttccgaaggtaactggcttcagcagagcgcagataccaaatactgttcttctagtgtagccgtagttaggccaccacttcaagaactctgtagcaccgcctacatacctcgctctgctaatcctgttaccagtggctgctgccagtggcgataagtcgtgtcttaccgggttggactcaagacgatagttaccggataaggcgcagcggtcgggctgaacggggggttcgtgcacacagcccagcttggagcgaacgacctacaccgaactgagatacctacagcgtgagctatgagaaagcgccacgcttcccgaagggagaaaggcggacaggtatccggtaagcggcagggtcggaacaggagagcgcacgagggagcttccagggggaaacgcctggtatctttatagtcctgtcgggtttcgccacctctgacttgagcgtcgatttttgtgatgctcgtcaggggggcggagcctatggaaaaacgccagcaacgcggcctttttacggttcctggccttttgctggccttttgctcacatgttctttcctgcgttatcccctgattctgtggataaccgtattaccgcctttgagtgagctgataccgctcgccgcagccgaacgaccgagcgcagcgagtcagtgagcgaggaagcggaagagcgcccaatacgcaaaccgcctctccccgcgcgttggccgattcattaatg

SEQ ID NO: 9 - DNA, 22 bp, Artificial Sequence
  Synthetic Primer
cagggctgggagctgggttctg

SEQ ID NO: 10 - DNA, 18 bp, Artificial Sequence
  Synthetic Primer
cccagggccttgatgcct

SEQ ID NO: 11 - DNA, 24 bp, Artificial Sequence
  Synthetic Primer
gctatcaggacatagcgttggcta